European Patent Specification EP 3 663 395 B1, published July 31, 2024. Title: NOVEL DELIVERY OF PACKAGED RNA TO MAMMALIAN CELLS. Applicant: THE UNITED STATES OF AMERICA, AS REPRESENTED BY THE SECRETARY, DEPARTMENT OF HEALTH AND HUMAN SERVICES. Application PCT/US13/31876. The sequence listing filed with the application follows.

SEQUENCE LISTING (1 sequence)

SEQ ID NO: 1 - DNA, 11913 bp, Artificial Sequence
  source: /note="Description of Artificial Sequence: Synthetic polynucleotide"
gacggatcgggagatctcccgatcccctatggtgcactctcagtacaatctgctctgatgccgcatagttaagccagtatctgctccctgcttgtgtgttggaggtcgctgagtagtgcgcgagcaaaatttaagctacaacaaggcaaggcttgaccgacaattgcatgaagaatctgcttagggttaggcgttttgcgctgcttcgcgatgtacgggccagatatacgcgttgacattgattattgactagttattaatagtaatcaattacggggtcattagttcatagcccatatatggagttccgcgttacataacttacggtaaatggcccgcctggctgaccgcccaacgacccccgcccattgacgtcaataatgacgtatgttcccatagtaacgccaatagggactttccattgacgtcaatgggtggagtatttacggtaaactgcccacttggcagtacatcaagtgtatcatatgccaagtacgccccctattgacgtcaatgacggtaaatggcccgcctggcattatgcccagtacatgaccttatgggactttcctacttggcagtacatctacgtattagtcatcgctattaccatggtgatgcggttttggcagtacatcaatgggcgtggatagcggtttgactcacggggatttccaagtctccaccccattgacgtcaatgggagtttgttttggcaccaaaatcaacgggactttccaaaatgtcgtaacaactccgccccattgacgcaaatgggcggtaggcgtgtacggtgggaggtctatataagcagagctcgtatggacatattgtcgttagaacgcggctacaattaatacataaccttatgtatcatacacatacgatttaggggacactatagattgacggcgtagtacacactattgaatcaaacagccgaccaattgcactaccatcacaatggagaagccagtagtaaacgtagacgtagacccccagagtccgtttgtcgtgcaactgcaaaaaagcttcccgcaatttgaggtagtagcacagcaggtcactccaaatgaccatgctaatgccagagcattttcgcatctggccagtaaactaatcgagctggaggttcctaccacagcgacgatcttggacataggcagcgcaccggctcgtagaatgttttccgagcaccagtatcattgtgtctgccccatgcgtagtccagaagacccggaccgcatgatgaaatacgccagtaaactggcggaaaaagcgtgcaagattacaaacaagaacttgcatgagaagattaaggatctccggaccgtacttgatacgccggatgctgaaacaccatcgctctgctttcacaacgatgttacctgcaacatgcgtgccgaatattccgtcatgcaggacgtgtatatcaacgctcccggaactatctatcatcaggctatgaaaggcgtgcggaccctgtactggattggcttcgacaccacccagttcatgttctcggctatggcaggttcgtaccctgcgtacaacaccaactgggccgacgagaaagtccttgaagcgcgtaacatcggactttgcagcacaaagctgagtgaaggtaggacaggaaaattgtcgataatgaggaagaaggagttgaagcccgggtcgcgggtttatttctccgtaggatcgacactttatccagaacacagagccagcttgcagagctggcatcttccatcggtgttccacttgaatggaaagcagtcgtacacttgccgctgtgatacagtggtgagttgcgaaggctacgtagtgaagaaaatcaccatcagtcccgggatcacgggagaaaccgtgggatacgcggttacacacaatagcgagggcttcttgctatgcaaagttactgacacagtaaaaggagaacgggtatcgttccctgtgtgcacgtacatcccggccaccatatgcgatcagatgactggtataatggccacggatatatcacctgacgatgcacaaaaacttctggttgggctcaaccagcgaattgtcattaacggtaggactaacaggaacaccaacaccatgcaaaattaccttctgccgatcatagcacaagggttcagcaaatgggctaaggagcgcaaggatgatcttgataacgagaaaatgctgggtactagagaacgcaagcttacgtatggctgcttgtgggcgtttcgcactaagaaagtacattcgttttatcgcccacctggaacgcagacctgcgtaaaagtcccagcctcttttagcgcttttcccatgtcgtccgtatggacgacctctttgcccatgtcgctgaggcagaaattgaaactggcattgcaaccaaagaaggaggaaaaactgctgcaggtctcggaggaattagtcatggaggccaaggctgcttttgaggatgctcaggaggaagccagagcggagaagctccgagaagcacttccaccattagtggcagacaaaggcatcgaggcagccgcagaagttgtctgcgaagtggaggggctccaggcggacatcggagcagcattagttgaaaccccgcgcggtcacgtaaggataatacctcaagcaaatgaccgtatgatcggacagtatatcgttgtctcgccaaactctgtgctgaagaatgccaaactcgcaccagcgcacccgctagcagatcaggttaagatcataacacactccggaagatcaggaaggtacgcggtcgaaccatacgacgctaaagtactgatgccagcaggaggtgccgtaccatggccagaattcctagcactgagtgagagcgccacgttagtgtacaacgaaagagagtttgtgaaccgcaaactataccacattgccatgcatggccccgccaagaatacagaagaggagcagtacaaggttacaaaggcagagcttgcagaaacagagtacgtgtttgacgtggacaagaagcgttgcgttaagaaggaagaagcctcaggtctggtcctctcgggagaactgaccaaccctccctatcatgagctagctctggagggactgaagacccgacctgcggtcccgtacaaggtcgaaacaataggagtgataggcacaccggggtcgggcaagtcagctattatcaagtcaactgtcacggcacgagatcttgttaccagcggaaagaaagaaaattgtcgcgaaattgaggccgacgtgctaagactgaggggtatgcagattacgtcgaagacagtagattcggttatgctcaacggatgccacaaagccgtagaagtgctgtacgttgacgaagcgttcgcgtgccacgcaggagcactacttgccttgattgctatcgtcaggccccgcaagaaggtagtactatgcggagaccccatgcaatgcggattcttcaacatgatgcaactaaaggtacatttcaatcaccctgaaaaagacatatgcaccaagacattctacaagtatatctcccggcgttgcacacagccagttacagctattgtatcgacactgcattacgatggaaagatgaaaaccacgaacccgtgcaagaagaacattgaaatcgatattacaggggccacaaagccgaagccaggggatatcatcctgacatgtttccgcgggtgggttaagcaattgcaaatcgactatcccggacatgaagtaatgacagccgcggcctcacaagggctaaccagaaaaggagtgtatgccgtccggcaaaaagtcaatgaaaacccactgtacgcgatcacatcagagcatgtgaacgtgttgctcacccgcactgaggacaggctagtgtggaaaaccttgcagggcgacccatggattaagcagcccactaacatacctaaaggaaactttcaggctactatagaggactgggaagctgaacacaagggaataattgctgcaataaacagccccactccccgtgccaatccgttcagctgcaagaccaacgtttgctgggcgaaagcattggaaccgatactagccacggccggtatcgtacttaccggttgccagtggagcgaactgttcccacagtttgcggatgacaaaccacattcggccatttacgccttagacgtaatttgcattaagtttttcggcatggacttgacaagcggactgttttctaaacagagcatcccactaacgtaccatcccgccgattcagcgaggccggtagctcattgggacaacagcccaggaacccgcaagtatgggtacgatcacgccattgccgccgaactctcccgtagatttccggtgttccagctagctgggaagggcacacaacttgatttgcagacggggagaaccagagttatctctgcacagcataacctggtcccggtgaaccgcaatcttcctcacgccttagtccccgagtacaaggagaagcaacccggcccggtcaaaaaattcttgaaccagttcaaacaccactcagtacttgtggtatcagaggaaaaaattgaagctccccgtaagagaatcgaatggatcgccccgattggcatagccggtgcagataagaactacaacctggctttcgggtttccgccgcaggcacggtacgacctggtgttcatcaacattggaactaaatacagaaaccaccactttcagcagtgcgaagaccatgcggcgaccttaaaaaccctttcgcgttcggccctgaattgccttaacccaggaggcaccctcgtggtgaagtcctatggctacgccgaccgcaacagtgaggacgtagtcaccgctcttgccagaaagtttgtcagggtgtctgcagcgagaccagattgtgtctcaagcaatacagaaatgtacctgattttccgacaactagacaacagccgtacacggcaattcaccccgcaccatctgaattgcgtgatttcgtccgtgtatgagggtacaagagatggagttggagccgcgccgtcataccgcaccaaaagggagaatattgctgactgtcaagaggaagcagttgtcaacgcagccaatccgctgggtagaccaggcgaaggagtctgccgtgccatctataaacgttggccgaccagttttaccgattcagccacggagacaggcaccgcaagaatgactgtgtgcctaggaaagaaagtgatccacgcggtcggccctgatttccggaagcacccagaagcagaagccttgaaattgctacaaaacgcctaccatgcagtggcagacttagtaaatgaacataacatcaagtctgtcgccattccactgctatctacaggcatttacgcagccggaaaagaccgccttgaagtatcacttaactgcttgacaaccgcgctagacagaactgacgcggacgtaaccatctattgcctggataagaagtggaaggaaagaatcgacgcggcactccaacttaaggagtctgtaacagagctgaaggatgaagatatggagatcgacgatgagttagtatggattcatccagacagttgcttgaagggaagaaagggattcagtactacaaaaggaaaattgtattcgtacttcgaaggcaccaaattccatcaagcagcaaaagacatggcggagataaaggtcctgttccctaatgaccaggaaagtaatgaacaactgtgtgcctacatattgggtgagaccatggaagcaatccgcgaaaagtgcccggtcgaccataacccgtcgtctagcccgcccaaaacgttgccgtgcctttgcatgtatgccatgacgccagaaagggtccacagacttagaagcaataacgtcaaagaagttacagtatgctcctccaccccccttcctaagcacaaaattaagaatgttcagaaggttcagtgcacgaaagtagtcctgtttaatccgcacactcccgcattcgttcccgcccgtaagtacatagaagtgccagaacagcctaccgctcctcctgcacaggccgaggaggcccccgaagttgtagcgacaccgtcaccatctacagctgataacacctcgcttgatgtcacagacatctcactggatatggatgacagtagcgaaggctcacttttttcgagctttagcggatcggacaactctattactagtatggacagttggtcgtcaggacctagttcactagagatagtagaccgaaggcaggtggtggtggctgacgttcatgccgtccaagagcctgcccctattccaccgccaaggctaaagaagatggcccgcctggcagcggcaagaaaagagcccactccaccggcaagcaatagctctgagtccctccacctctcttttggtggggtatccatgtccctcggatcaattttcgacggagagacggcccgccaggcagcggtacaacccctggcaacaggccccacggatgtgcctatgtctttcggatcgttttccgacggagagattgatgagctgagccgcagagtaactgagtccgaacccgtcctgtttggatcatttgaaccgggcgaagtgaactcaattatatcgtcccgatcagccgtatcttttccactacgcaagcagagacgtagacgcaggagcaggaggactgaatactgactaaccggggtaggtgggtacatattttcgacggacacaggccctgggcacttgcaaaagaagtccgttctgcagaaccagcttacagaaccgaccttggagcgcaatgtcctggaaagaattcatgccccggtgctcgacacgtcgaaagaggaacaactcaaactcaggtaccagatgatgcccaccgaagccaacaaaagtaggtaccagtctcgtaaagtagaaaatcagaaagccataaccactgagcgactactgtcaggactacgactgtataactctgccacagatcagccagaatgctataagatcacctatccgaaaccattgtactccagtagcgtaccggcgaactactccgatccacagttcgctgtagctgtctgtaacaactatctgcatgagaactatccgacagtagcatcttatcagattactgacgagtacgatgcttacttggatatggtagacgggacagtcgcctgcctggatactgcaaccttctgccccgctaagcttagaagttacccgaaaaaacatgagtatagagccccgaatatccgcagtgcggttccatcagcgatgcagaacacgctacaaaatgtgctcattgccgcaactaaaagaaattgcaacgtcacgcagatgcgtgaactgccaacactggactcagcgacattcaatgtcgaatgctttcgaaaatatgcatgtaatgacgagtattgggaggagttcgctcggaagccaattaggattaccactgagtttgtcaccgcatatgtagctagactgaaaggccctaaggccgccgcactatttgcaaagacgtataatttggtcccattgcaagaagtgcctatggatagattcgtcatggacatgaaaagagacgtgaaagttacaccaggcacgaaacacacagaagaaagaccgaaagtacaagtgatacaagccgcagaacccctggcgactgcttacttatgcgggattcaccgggaattagtgcgtaggcttacggccgtcttgcttccaaacattcacacgctttttgacatgtcggcggaggattttgatgcaatcatagcagaacacttcaagcaaggcgacccggtactggagacggatatcgcatcattcgacaaaagccaagacgacgctatggcgttaaccggtctgatgatcttggaggacctgggtgtggatcaaccactactcgacttgatcgagtgcgcctttggagaaatatcatccacccatctacctacgggtactcgttttaaattcggggcgatgatgaaatccggaatgttcctcacactttttgtcaacacagttttgaatgtcgttatcgccagcagagtactagaagagcggcttaaaacgtccagatgtgcagcgttcattggcgacgacaacatcatacatggagtagtatctgacaaagaaatggctgagaggtgcgccacctggctcaacatggaggttaagatcatcgacgcagtcatcggtgagagaccaccttacttctgcggcggatttatcttgcaagattcggttacttccacagcgtgccgcgtggcggatcccctgaaaaggctgtttaagttgggtaaaccgctcccagccgacgacgagcaagacgaagacagaagacgcgctctgctagatgaaacaaaggcgtggtttagagtaggtataacaggcactttagcagtggccgtgacgacccggtatgaggtagacaatattacacctgtcctactggcattgagaacttttgcccagagcaaaagagcattccaagccatcagaggggaaataaagcatctctacggtggtcctaaatagtcagcatagtacatttcatctgactaatactacaacaccaccacctctagagcttgccgccaccatggtgagcaagggcgaggagctgttcaccggggtggtgcccatcctggtcgagctggacggcgacgtgaacggccacaagttcagcgtgtccggcgagggcgagggcgatgccacctacggcaagctgaccctgaagttcatctgcaccaccggcaagctgcccgtgccctggcccaccctcgtgaccaccctgacctacggcgtgcagtgcttcagccgctaccccgaccacatgaagcagcacgacttcttcaagtccgccatgcccgaaggctacgtccaggagcgcaccatcttcttcaaggacgacggcaactacaagacccgcgccgaggtgaagttcgagggcgacaccctggtgaaccgcatcgagctgaagggcatcgacttcaaggaggacggcaacatcctggggcacaagctggagtacaactacaacagccacaacgtctatatcatggccgacaagcagaagaacggcatcaaggtgaacttcaagatccgccacaacatcgaggacggcagcgtgcagctcgccgaccactaccagcagaacacccccatcggcgacggccccgtgctgctgcccgacaaccactacctgagcacccagtccgccctgagcaaagaccccaacgagaagcgcgatcacatggtcctgctggagttcgtgaccgccgccgggatcactcacggcatggacgagctgtacaagtaaagcggccgtgagcatgcaggccttgggcccaatgatccgaccagcaaaactcgatgtacttccgaggaactgatgtgcataatgcatcaggctggtacattagatccccgcttaccgcgggcaatatagcaacactaaaaactcgatgtacttccgaggaagcgcagtgcataatgctgcgcagtgttgccacataaccactatattaaccatttatctagcggacgccaaaaactcaatgtatttctgaggaagcgtggtgcataatgccacgcagcgtctgcataacttttattatttcttttattaatcaacaaaattttgtttttaacatttcaaaaaaaaaaaaaaaaaaaaaaaaaaaaaaaaaaaaagggaattcctcgattaattaagcggccgctcgagatggcacacgtgttacggttttaccgtcgacctctagctagagcttggcgtaatcatggtcatagctgtttcctgtgtgaaattgttatccgctcacaattccacacaacatacgagccggaagcataaagtgtaaagcctggggtgcctaatgagtgagctaactcacattaattgcgttgcgctcactgcccgctttccagtcgggaaacctgtcgtgccagctgcattaatgaatcggccaacgcgcggggagaggcggtttgcgtattgggcgctcttccgcttcctcgctcactgactcgctgcgctcggtcgttcggctgcggcgagcggtatcagctcactcaaaggcggtaatacggttatccacagaatcaggggataacgcaggaaagaacatgtgagcaaaaggccagcaaaaggccaggaaccgtaaaaaggccgcgttgctggcgtttttccataggctccgcccccctgacgagcatcacaaaaatcgacgctcaagtcagaggtggcgaaacccgacaggactataaagataccaggcgtttccccctggaagctccctcgtgcgctctcctgttccgaccctgccgcttaccggatacctgtccgcctttctcccttcgggaagcgtggcgctttctcatagctcacgctgtaggtatctcagttcggtgtaggtcgttcgctccaagctgggctgtgtgcacgaaccccccgttcagcccgaccgctgcgccttatccggtaactatcgtcttgagtccaacccggtaagacacgacttatcgccactggcagcagccactggtaacaggattagcagagcgaggtatgtaggcggtgctacagagttcttgaagtggtggcctaactacggctacactagaagaacagtatttggtatctgcgctctgctgaagccagttaccttcggaaaaagagttggtagctcttgatccggcaaacaaaccaccgctggtagcggtggtttttttgtttgcaagcagcagattacgcgcagaaaaaaaggatctcaagaagatcctttgatcttttctacggggtctgacgctcagtggaacgaaaactcacgttaagggattttggtcatgagattatcaaaaaggatcttcacctagatccttttaaattaaaaatgaagttttaaatcaatctaaagtatatatgagtaaacttggtctgacagttaccaatgcttaatcagtgaggcacctatctcagcgatctgtctatttcgttcatccatagttgcctgactccccgtcgtgtagataactacgatacgggagggcttaccatctggccccagtgctgcaatgataccgcgagacccacgctcaccggctccagatttatcagcaataaaccagccagccggaagggccgagcgcagaagtggtcctgcaactttatccgcctccatccagtctattaattgttgccgggaagctagagtaagtagttcgccagttaatagtttgcgcaacgttgttgccattgctacaggcatcgtggtgtcacgctcgtcgtttggtatggcttcattcagctccggttcccaacgatcaaggcgagttacatgatcccccatgttgtgcaaaaaagcggttagctccttcggtcctccgatcgttgtcagaagtaagttggccgcagtgttatcactcatggttatggcagcactgcataattctcttactgtcatgccatccgtaagatgcttttctgtgactggtgagtactcaaccaagtcattctgagaatagtgtatgcggcgaccgagttgctcttgcccggcgtcaatacgggataataccgcgccacatagcagaactttaaaagtgctcatcattggaaaacgttcttcggggcgaaaactctcaaggatcttaccgctgttgagatccagttcgatgtaacccactcgtgcacccaactgatcttcagcatcttttactttcaccagcgtttctgggtgagcaaaaacaggaaggcaaaatgccgcaaaaaagggaataagggcgacacggaaatgttgaatactcatactcttcctttttcaatattattgaagcatttatcagggttattgtctcatgagcggatacatatttgaatgtatttagaaaaataaacaaataggggttccgcgcacatttccccgaaaagtgccacctgacgtc